European Patent Application EP 4 534 108 A1, published April 9, 2025. Title: Composition comprising anionic long-chain fatty acid for use in attenuating skin barrier function and dispersion dispersing complexes comprising cationic long-chain lipid and anionic long-chain lipid and drug. Applicant: Kyushu University. The sequence listing filed with the application follows.

SEQUENCE LISTING (2 sequences)

SEQ ID NO: 1 - DNA, 17 bp, synthetic construct
  source 1..17: mol_type = other DNA
cggcatgtctatttgta

SEQ ID NO: 2 - DNA, 14 bp, synthetic construct
  misc_feature 4..10: note = DNA
  source 1..14: mol_type = other DNA
  misc_feature 14: note = DNA
  modified_base 1..3: mod_base = OTHER; note = LNA
  modified_base 11..13: mod_base = OTHER; note = LNA
  modified_base 11: mod_base = cm
  modified_base 13: mod_base = cm
  modified_base 1..14: mod_base = OTHER; note = phosphorothioate
gaaacctatgcaca